European Patent Application EP 4 538 289 A1, published April 16, 2025. Title: CD73 ANTIBODY COCKTAIL THERAPY. Applicant: 上海华奥泰生物药业股份有限公司. The sequence listing filed with the application follows.

SEQUENCE LISTING (38 sequences)

SEQ ID NO: 1 - protein, 18 aa, synthetic construct
  REGION 1..18: note = 900698 HCDR3
ARAIYYYGSSYNYYAMDY

SEQ ID NO: 2 - protein, 8 aa, synthetic construct
  REGION 1..8: note = 900698 HCDR2
ISSGGGYI

SEQ ID NO: 3 - protein, 8 aa, synthetic construct
  REGION 1..8: note = 900698 HCDR1
GFTFSKYA

SEQ ID NO: 4 - protein, 25 aa, synthetic construct
  REGION 1..25: note = 900698 H-FR1
QVQLVESGGGLVKPGGSLRLSCAAS

SEQ ID NO: 5 - protein, 17 aa, synthetic construct
  REGION 1..17: note = 900698 H-FR2
MSWIRQAPGKGLEWVAE

SEQ ID NO: 6 - protein, 38 aa, synthetic construct
  REGION 1..38: note = 900698 H-FR3
NYADSVKGRFTISRDNAKNSLYLQMNSLRAEDTAVYYC

SEQ ID NO: 7 - protein, 11 aa, synthetic construct
  REGION 1..11: note = 900698/900725 H-FR4
WGQGTTVTVSS

SEQ ID NO: 8 - protein, 125 aa, synthetic construct
  REGION 1..125: note = 900698 VH
QVQLVESGGGLVKPGGSLRLSCAASGFTFSKYAMSWIRQAPGKGLEWVAEISSGGGYINYADSVKGRFTISRDNAKNSLYLQMNSLRAEDTAVYYCARAIYYYGSSYNYYAMDYWGQGTTVTVSS

SEQ ID NO: 9 - protein, 329 aa, synthetic construct
  REGION 1..329: note = 900698/900725 heavy chain constant region
ASTKGPSVFPLAPSSKSTSGGTAALGCLVKDYFPEPVTVSWNSGALTSGVHTFPAVLQSSGLYSLSSVVTVPSSSLGTQTYICNVNHKPSNTKVDKRVEPKSCDKTHTCPPCPAPEAAGGPSVFLFPPKPKDTLMISRTPEVTCVVVDVSHEDPEVKFNWYVDGVEVHNAKTKPREEQYNSTYRVVSVLTVLHQDWLNGKEYKCKVSNKALPAPIEKTISKAKGQPREPQVYTLPPSREEMTKNQVSLTCLVKGFYPSDIAVEWESNGQPENNYKTTPPVLDSDGSFFLYSKLTVDKSRWQQGNVFSCSVMHEALHNHYTQKSLSLSPG

SEQ ID NO: 10 - protein, 454 aa, synthetic construct
  REGION 1..454: note = 900698 heavy chain
QVQLVESGGGLVKPGGSLRLSCAASGFTFSKYAMSWIRQAPGKGLEWVAEISSGGGYINYADSVKGRFTISRDNAKNSLYLQMNSLRAEDTAVYYCARAIYYYGSSYNYYAMDYWGQGTTVTVSSASTKGPSVFPLAPSSKSTSGGTAALGCLVKDYFPEPVTVSWNSGALTSGVHTFPAVLQSSGLYSLSSVVTVPSSSLGTQTYICNVNHKPSNTKVDKRVEPKSCDKTHTCPPCPAPEAAGGPSVFLFPPKPKDTLMISRTPEVTCVVVDVSHEDPEVKFNWYVDGVEVHNAKTKPREEQYNSTYRVVSVLTVLHQDWLNGKEYKCKVSNKALPAPIEKTISKAKGQPREPQVYTLPPSREEMTKNQVSLTCLVKGFYPSDIAVEWESNGQPENNYKTTPPVLDSDGSFFLYSKLTVDKSRWQQGNVFSCSVMHEALHNHYTQKSLSLSPG

SEQ ID NO: 11 - protein, 9 aa, synthetic construct
  REGION 1..9: note = 900698 LCDR3
QQYSSYPLT

SEQ ID NO: 12 - skipped

SEQ ID NO: 13 - protein, 6 aa, synthetic construct
  REGION 1..6: note = 900698 LCDR1
QDVGTA

SEQ ID NO: 14 - protein, 26 aa, synthetic construct [sequence omitted]

SEQ ID NO: 15 - protein, 17 aa, synthetic construct
  REGION 1..17: note = 900698 L-FR2
EAWYQQKPGKAPKLLIY

SEQ ID NO: 16 - protein, 36 aa, synthetic construct
  REGION 1..36: note = 900698 L-FR3
TRHTGVPSRFSGSGSGTDFTLTISSLQPEDFATYYC

SEQ ID NO: 17 - protein, 10 aa, synthetic construct
  REGION 1..10: note = 900698/900725 L-FR4
FGQGTKLEIK

SEQ ID NO: 18 - protein, 107 aa, synthetic construct
  REGION 1..107: note = 900698 VL
DIQMTQSPSSLSASVGDRVTITCRASQDVGTAEAWYQQKPGKAPKLLIYWASTRHTGVPSRFSGSGSGTDFTLTISSLQPEDFATYYCQQYSSYPLTFGQGTKLEIK

SEQ ID NO: 19 - protein, 107 aa, synthetic construct [sequence omitted]

SEQ ID NO: 20 - protein, 214 aa, synthetic construct
  REGION 1..214: note = 900698 light chain
DIQMTQSPSSLSASVGDRVTITCRASQDVGTAEAWYQQKPGKAPKLLIYWASTRHTGVPSRFSGSGSGTDFTLTISSLQPEDFATYYCQQYSSYPLTFGQGTKLEIKRTVAAPSVFIFPPSDEQLKSGTASVVCLLNNFYPREAKVQWKVDNALQSGNSQESVTEQDSKDSTYSLSSTLTLSKADYEKHKVYACEVTHQGLSSPVTKSFNRGEC

SEQ ID NO: 21 - protein, 14 aa, synthetic construct
  REGION 1..14: note = 900725 HCDR3
ARYYGSDYEWYFDV

SEQ ID NO: 22 - protein, 8 aa, synthetic construct
  REGION 1..8: note = 900725 HCDR2
IHPNSGST

SEQ ID NO: 23 - protein, 8 aa, synthetic construct
  REGION 1..8: note = 900725 HCDR1
GYTFTSYW

SEQ ID NO: 24 - protein, 25 aa, synthetic construct
  REGION 1..25: note = 900725 H-FR1
QVQLVQSGAEVKKPGASVKLSCKAS

SEQ ID NO: 25 - protein, 17 aa, synthetic construct
  REGION 1..17: note = 900725 H-FR2
IHWVRQAPGQGLEWIGM

SEQ ID NO: 26 - protein, 38 aa, synthetic construct
  REGION 1..38: note = 900725 H-FR3
YYNEKFKGRATLTVDKSTSTAYMELSSLRSEDTAVYYC

SEQ ID NO: 27 - protein, 121 aa, synthetic construct
  REGION 1..121: note = 900725 VH
QVQLVQSGAEVKKPGASVKLSCKASGYTFTSYWIHWVRQAPGQGLEWIGMIHPNSGSTYYNEKFKGRATLTVDKSTSTAYMELSSLRSEDTAVYYCARYYGSDYEWYFDVWGQGTTVTVSS

SEQ ID NO: 28 - protein, 450 aa, synthetic construct
  REGION 1..450: note = 900725 heavy chain
QVQLVQSGAEVKKPGASVKLSCKASGYTFTSYWIHWVRQAPGQGLEWIGMIHPNSGSTYYNEKFKGRATLTVDKSTSTAYMELSSLRSEDTAVYYCARYYGSDYEWYFDVWGQGTTVTVSSASTKGPSVFPLAPSSKSTSGGTAALGCLVKDYFPEPVTVSWNSGALTSGVHTFPAVLQSSGLYSLSSVVTVPSSSLGTQTYICNVNHKPSNTKVDKRVEPKSCDKTHTCPPCPAPEAAGGPSVFLFPPKPKDTLMISRTPEVTCVVVDVSHEDPEVKFNWYVDGVEVHNAKTKPREEQYNSTYRVVSVLTVLHQDWLNGKEYKCKVSNKALPAPIEKTISKAKGQPREPQVYTLPPSREEMTKNQVSLTCLVKGFYPSDIAVEWESNGQPENNYKTTPPVLDSDGSFFLYSKLTVDKSRWQQGNVFSCSVMHEALHNHYTQKSLSLSPG

SEQ ID NO: 29 - protein, 9 aa, synthetic construct
  REGION 1..9: note = 900725 LCDR3
LQHWNYPYT

SEQ ID NO: 30 - skipped

SEQ ID NO: 31 - protein, 6 aa, synthetic construct
  REGION 1..6: note = 900725 LCDR1
QNVRTA

SEQ ID NO: 32 - protein, 26 aa, synthetic construct
  REGION 1..26: note = 900725 L-FR1
DIQMTQSPSSMSASVGDRVTITCKAS

SEQ ID NO: 33 - protein, 17 aa, synthetic construct
  REGION 1..17: note = 900725 L-FR2
VVWYQQKPGKAPKALIY

SEQ ID NO: 34 - protein, 36 aa, synthetic construct
  REGION 1..36: note = 900725 L-FR3
NRHTGVPDRFSGSGSGTDFTLTISSLQPEDFATYFC

SEQ ID NO: 35 - protein, 107 aa, synthetic construct
  REGION 1..107: note = 900725 VL
DIQMTQSPSSMSASVGDRVTITCKASQNVRTAVVWYQQKPGKAPKALIYLASNRHTGVPDRFSGSGSGTDFTLTISSLQPEDFATYFCLQHWNYPYTFGQGTKLEIK

SEQ ID NO: 36 - protein, 214 aa, synthetic construct
  REGION 1..214: note = 900725 light chain
DIQMTQSPSSMSASVGDRVTITCKASQNVRTAVVWYQQKPGKAPKALIYLASNRHTGVPDRFSGSGSGTDFTLTISSLQPEDFATYFCLQHWNYPYTFGQGTKLEIKRTVAAPSVFIFPPSDEQLKSGTASVVCLLNNFYPREAKVQWKVDNALQSGNSQESVTEQDSKDSTYSLSSTLTLSKADYEKHKVYACEVTHQGLSSPVTKSFNRGEC

SEQ ID NO: 37 - protein, 450 aa, synthetic construct
  REGION 1..450: note = 900201 heavy chain
QIQLVQSGPELKKPGETVKISCKTSGYTFTNYGMNWVKQAPGKGLKWVGWINTYTGEPKYADDFKGRFAFSVETSASTAYLQINNLKNEDTATYFCARGIYDGYHWYFDVWGAGTTVTVSSASTKGPSVFPLAPSSKSTSGGTAALGCLVKDYFPEPVTVSWNSGALTSGVHTFPAVLQSSGLYSLSSVVTVPSSSLGTQTYICNVNHKPSNTKVDKRVEPKSCDKTHTCPPCPAPELLGGPSVFLFPPKPKDTLMISRTPEVTCVVVDVSHEDPEVKFNWYVDGVEVHNAKTKPREEQYNSTYRVVSVLTVLHQDWLNGKEYKCKVSNKALPAPIEKTISKAKGQPREPQVYTLPPSREEMTKNQVSLTCLVKGFYPSDIAVEWESNGQPENNYKTTPPVLDSDGSFFLYSKLTVDKSRWQQGNVFSCSVMHEALHNHYTQKSLSLSPG

SEQ ID NO: 38 - protein, 219 aa, synthetic construct
  REGION 1..219: note = 900201 light chain
DVVMTQTPLSLPVSLGDQASISCRSSQSLVHSIGNTYLHWYLQKPGQSPKLLIYKVSNRFSGVPDRFSGSGSGTDFTLKITRVEAEDLGVYFCSQSTHVPFTFGSGTKLEIKRTVAAPSVFIFPPSDEQLKSGTASVVCLLNNFYPREAKVQWKVDNALQSGNSQESVTEQDSKDSTYSLSSTLTLSKADYEKHKVYACEVTHQGLSSPVTKSFNRGEC